European Patent Application EP 4 223 125 A2, published August 9, 2023. Title: METHODS AND COMPOSITIONS FOR REARING PREDATOR INSECTS. Applicant: AGROBÍO, S.L. The sequence listing filed with the application follows.

SEQUENCE LISTING (2 sequences)

SEQ ID NO: 1 - DNA, 23 bp, synthetic construct
  source 1..23: mol_type = other DNA; note = RP02 Forward primer
tacacactttgccgtaaatcaga

SEQ ID NO: 2 - DNA, 22 bp, synthetic construct
  source 1..22: mol_type = other DNA; note = RP02 Reverse primer
cgttgtattggcatgatatagg